European Patent Specification EP 3 360 886 B1, published January 25, 2023. Title: FOXM1 PEPTIDES AND VACCINES COMPRISING THE SAME. Applicant: ONCOTHERAPY SCIENCE,INC. The sequence listing filed with the application follows.

SEQUENCE LISTING (76 sequences)

SEQ ID NO: 1 - protein, 9 aa, Artificial Sequence
  a peptide derived from FOXM1
SLSNIQWLR

SEQ ID NO: 2 - protein, 9 aa, Artificial Sequence
  a peptide derived from FOXM1
WTIHPSANR

SEQ ID NO: 3 - protein, 9 aa, Artificial Sequence
  a peptide derived from FOXM1
QVSGLAANR

SEQ ID NO: 4 - protein, 9 aa, Artificial Sequence
  a peptide derived from FOXM1
MSSDGLGSR

SEQ ID NO: 5 - protein, 9 aa, Artificial Sequence
  a peptide derived from FOXM1
MLVIQHRER

SEQ ID NO: 6 - protein, 9 aa, Artificial Sequence
  a peptide derived from FOXM1
LVIQHRERR

SEQ ID NO: 7 - protein, 9 aa, Artificial Sequence
  a peptide derived from FOXM1
AARDVNLPR

SEQ ID NO: 8 - protein, 9 aa, Artificial Sequence
  a peptide derived from FOXM1
TLGPKPAAR

SEQ ID NO: 9 - protein, 9 aa, Artificial Sequence
  a peptide derived from FOXM1
SLMSSELAR

SEQ ID NO: 10 - protein, 9 aa, Artificial Sequence
  a peptide derived from FOXM1
QFAINSTER

SEQ ID NO: 11 - protein, 9 aa, Artificial Sequence
  a peptide derived from FOXM1
LSLHDMFVR

SEQ ID NO: 12 - protein, 9 aa, Artificial Sequence
  a peptide derived from FOXM1
SWQNSVSER

SEQ ID NO: 13 - protein, 9 aa, Artificial Sequence
  a peptide derived from FOXM1
TQTSYDAKR

SEQ ID NO: 14 - protein, 9 aa, Artificial Sequence
  a peptide derived from FOXM1
DSSQSPTPR

SEQ ID NO: 15 - protein, 9 aa, Artificial Sequence
  a peptide derived from FOXM1
FPYFKHIAK

SEQ ID NO: 16 - protein, 9 aa, Artificial Sequence
  a peptide derived from FOXM1
QVKVEEPSR

SEQ ID NO: 17 - protein, 9 aa, Artificial Sequence
  a peptide derived from FOXM1
YSGLRSPTR

SEQ ID NO: 18 - protein, 9 aa, Artificial Sequence
  a peptide derived from FOXM1
DQVFKQQKR

SEQ ID NO: 19 - protein, 9 aa, Artificial Sequence
  a peptide derived from FOXM1
SELARHSKR

SEQ ID NO: 20 - protein, 9 aa, Artificial Sequence
  a peptide derived from FOXM1
KTELPLGAR

SEQ ID NO: 21 - protein, 9 aa, Artificial Sequence
  a peptide derived from FOXM1
FSEGPSTSR

SEQ ID NO: 22 - protein, 10 aa, Artificial Sequence
  a peptide derived from FOXM1
EMLVIQHRER

SEQ ID NO: 23 - protein, 10 aa, Artificial Sequence
  a peptide derived from FOXM1
ETLGPKPAAR

SEQ ID NO: 24 - protein, 10 aa, Artificial Sequence
  a peptide derived from FOXM1
NSLSNIQWLR

SEQ ID NO: 25 - protein, 10 aa, Artificial Sequence
  a peptide derived from FOXM1
NLSLHDMFVR

SEQ ID NO: 26 - protein, 10 aa, Artificial Sequence
  a peptide derived from FOXM1
SYSGLRSPTR

SEQ ID NO: 27 - protein, 10 aa, Artificial Sequence
  a peptide derived from FOXM1
MLVIQHRERR

SEQ ID NO: 28 - protein, 10 aa, Artificial Sequence
  a peptide derived from FOXM1
FWTIHPSANR

SEQ ID NO: 29 - protein, 10 aa, Artificial Sequence
  a peptide derived from FOXM1
HSKRVRIAPK

SEQ ID NO: 30 - protein, 10 aa, Artificial Sequence
  a peptide derived from FOXM1
IQFAINSTER

SEQ ID NO: 31 - protein, 10 aa, Artificial Sequence
  a peptide derived from FOXM1
HFPYFKHIAK

SEQ ID NO: 32 - protein, 10 aa, Artificial Sequence
  a peptide derived from FOXM1
QTQTSYDAKR

SEQ ID NO: 33 - protein, 10 aa, Artificial Sequence
  a peptide derived from FOXM1
STPSKSVLPR

SEQ ID NO: 34 - protein, 10 aa, Artificial Sequence
  a peptide derived from FOXM1
ELARHSKRVR

SEQ ID NO: 35 - protein, 10 aa, Artificial Sequence
  a peptide derived from FOXM1
FAINSTERKR

SEQ ID NO: 36 - protein, 10 aa, Artificial Sequence
  a peptide derived from FOXM1
LFSEGPSTSR

SEQ ID NO: 37 - protein, 10 aa, Artificial Sequence
  a peptide derived from FOXM1
SSELARHSKR

SEQ ID NO: 38 - protein, 10 aa, Artificial Sequence
  a peptide derived from FOXM1
ASWQNSVSER

SEQ ID NO: 39 - protein, 10 aa, Artificial Sequence
  a peptide derived from FOXM1
MSSELARHSK

SEQ ID NO: 40 - protein, 10 aa, Artificial Sequence
  a peptide derived from FOXM1
QQKRPNPELR

SEQ ID NO: 41 - protein, 10 aa, Artificial Sequence
  a peptide derived from FOXM1
ESWRLTPPAK

SEQ ID NO: 42 - protein, 10 aa, Artificial Sequence
  a peptide derived from FOXM1
WIEDHFPYFK

SEQ ID NO: 43 - protein, 10 aa, Artificial Sequence
  a peptide derived from FOXM1
RPKKSYSGLR

SEQ ID NO: 44 - protein, 10 aa, Artificial Sequence
  a peptide derived from FOXM1
EWPSPAPSFK

SEQ ID NO: 45 - protein, 10 aa, Artificial Sequence
  a peptide derived from FOXM1
SPRRPLILKR

SEQ ID NO: 46 - protein, 10 aa, Artificial Sequence
  a peptide derived from FOXM1
ASLMSSELAR

SEQ ID NO: 47 - protein, 10 aa, Artificial Sequence
  a peptide derived from FOXM1
SAPPLESPQR

SEQ ID NO: 48 - protein, 9 aa, Artificial Sequence
  a peptide derived from FOXM1
VSERPPYSY

SEQ ID NO: 49 - protein, 9 aa, Artificial Sequence
  a peptide derived from FOXM1
CVDEPELLF

SEQ ID NO: 50 - protein, 9 aa, Artificial Sequence
  a peptide derived from FOXM1
ASDPLPDPL

SEQ ID NO: 51 - protein, 9 aa, Artificial Sequence
  a peptide derived from FOXM1
LTEGLVLDT

SEQ ID NO: 52 - protein, 9 aa, Artificial Sequence
  a peptide derived from FOXM1
NSVSERPPY

SEQ ID NO: 53 - protein, 9 aa, Artificial Sequence
  a peptide derived from FOXM1
SSEPLDLIS

SEQ ID NO: 54 - protein, 9 aa, Artificial Sequence
  a peptide derived from FOXM1
SSELARHSK

SEQ ID NO: 55 - protein, 9 aa, Artificial Sequence
  a peptide derived from FOXM1
PTPRPKKSY

SEQ ID NO: 56 - protein, 10 aa, Artificial Sequence
  a peptide derived from FOXM1
SSDPASQLSY

SEQ ID NO: 57 - protein, 10 aa, Artificial Sequence
  a peptide derived from FOXM1
YTWIEDHFPY

SEQ ID NO: 58 - protein, 10 aa, Artificial Sequence
  a peptide derived from FOXM1
WTIHPSANRY

SEQ ID NO: 59 - protein, 10 aa, Artificial Sequence
  a peptide derived from FOXM1
SVSERPPYSY

SEQ ID NO: 60 - protein, 10 aa, Artificial Sequence
  a peptide derived from FOXM1
SSEPLDLISV

SEQ ID NO: 61 - protein, 10 aa, Artificial Sequence
  a peptide derived from FOXM1
KTELPLGARR

SEQ ID NO: 62 - DNA, 22 bp, Artificial Sequence
  a PCR primer for the TCR analysis
gtctaccaggcattcgcttcat

SEQ ID NO: 63 - DNA, 24 bp, Artificial Sequence
  a PCR primer for the TCR analysis
tcagctggaccacagccgcagcgt

SEQ ID NO: 64 - DNA, 21 bp, Artificial Sequence
  a PCR primer for the TCR analysis
tcagaaatcctttctcttgac

SEQ ID NO: 65 - DNA, 24 bp, Artificial Sequence
  a PCR primer for the TCR analysis
ctagcctctggaatcctttctctt

SEQ ID NO: 66 - DNA, 3506 bp, Homo sapiens
  CDS (284)..(2530)
tttcaaacagcggaacaaactgaaagctccggtgccagaccccacccccggccccggcccgggaccccctcccctcccgggatcccccggggttcccaccccgcccgcaccgccggggacccggccggtccggcgcgagcccccgtccggggccctggctcggcccccaggttggaggagcccggagcccgccttcggagctacggcctaacggcggcggcgactgcagtctggagggtccacacttgtgattctcaatggagagtgaaaacgcagattcataatgaaaactagcccccgtcggccactgattctcaaaagacggaggctgccccttcctgttcaaaatgccccaagtgaaacatcagaggaggaacctaagagatcccctgcccaacaggagtctaatcaagcagaggcctccaaggaagtggcagagtccaactcttgcaagtttccagctgggatcaagattattaaccaccccaccatgcccaacacgcaagtagtggccatccccaacaatgctaatattcacagcatcatcacagcactgactgccaagggaaaagagagtggcagtagtgggcccaacaaattcatcctcatcagctgtgggggagccccaactcagcctccaggactccggcctcaaacccaaaccagctatgatgccaaaaggacagaagtgaccctggagaccttgggaccaaaacctgcagctagggatgtgaatcttcctagaccacctggagccctttgcgagcagaaacgggagacctgtgcagatggtgaggcagcaggctgcactatcaacaatagcctatccaacatccagtggcttcgaaagatgagttctgatggactgggctcccgcagcatcaagcaagagatggaggaaaaggagaattgtcacctggagcagcgacaggttaaggttgaggagccttcgagaccatcagcgtcctggcagaactctgtgtctgagcggccaccctactcttacatggccatgatacaattcgccatcaacagcactgagaggaagcgcatgactttgaaagacatctatacgtggattgaggaccactttccctactttaagcacattgccaagccaggctggaagaactccatccgccacaacctttccctgcacgacatgtttgtccgggagacgtctgccaatggcaaggtctccttctggaccattcaccccagtgccaaccgctacttgacattggaccaggtgtttaagcagcagaaacgaccgaatccagagctccgccggaacatgaccatcaaaaccgaactccccctgggcgcacggcggaagatgaagccactgctaccacgggtcagctcatacctggtacctatccagttcccggtgaaccagtcactggtgttgcagccctcggtgaaggtgccattgcccctggcggcttccctcatgagctcagagcttgcccgccatagcaagcgagtccgcattgcccccaaggtgctgctagctgaggaggggatagctcctctttcttctgcaggaccagggaaagaggagaaactcctgtttggagaagggttttctcctttgcttccagttcagactatcaaggaggaagaaatccagcctggggaggaaatgccacacttagcgagacccatcaaagtggagagccctcccttggaagagtggccctccccggccccatctttcaaagaggaatcatctcactcctgggaggattcgtcccaatctcccaccccaagacccaagaagtcctacagtgggcttaggtccccaacccggtgtgtctcggaaatgcttgtgattcaacacagggagaggagggagaggagccggtctcggaggaaacagcatctactgcctccctgtgtggatgagccggagctgctcttctcagaggggcccagtacttcccgctgggccgcagagctcccgttcccagcagactcctctgaccctgcctcccagctcagctactcccaggaagtgggaggaccttttaagacacccattaaggaaacgctgcccatctcctccaccccgagcaaatctgtcctccccagaacccctgaatcctggaggctcacgcccccagccaaagtagggggactggatttcagcccagtacaaacctcccagggtgcctctgaccccttgcctgaccccctggggctgatggatctcagcaccactcccttgcaaagtgctcccccccttgaatcaccgcaaaggctcctcagttcagaacccttagacctcatctccgtcccctttggcaactcttctccctcagatatagacgtccccaagccaggctccccggagccacaggtttctggccttgcagccaatcgttctctgacagaaggcctggtcctggacacaatgaatgacagcctcagcaagatcctgctggacatcagctttcctggcctggacgaggacccactgggccctgacaacatcaactggtcccagtttattcctgagctacagtagagccctgcccttgcccctgtgctcaagctgtccaccatcccgggcactccaaggctcagtgcaccccaagcctctgagtgaggacagcaggcagggactgttctgctcctcatagctccctgctgcctgattatgcaaaagtagcagtcacaccctagccactgctgggaccttgtgttccccaagagtatctgattcctctgctgtccctgccaggagctgaagggtgggaacaacaaaggcaatggtgaaaagagattaggaaccccccagcctgtttccattctctgcccagcagtctcttaccttccctgatctttgcagggtggtccgtgtaaatagtataaattctccaaattatcctctaattataaatgtaagcttatttccttagatcattatccagagactgccagaaggtgggtaggatgacctggggtttcaattgacttctgttccttgcttttagttttgatagaagggaagacctgcagtgcacggtttcttccaggctgaggtacctggatcttgggttcttcactgcagggacccagacaagtggatctgcttgccagagtcctttttgcccctccctgccacctccccgtgtttccaagtcagctttcctgcaagaagaaatcctggttaaaaaagtcttttgtattgggtcaggagttgaatttggggtgggaggatggatgcaactgaagcagagtgtgggtgcccagatgtgcgctattagatgtttctctgataatgtccccaatcataccagggagactggcattgacgagaactcaggtggaggcttgagaaggccgaaagggcccctgacctgcctggcttccttagcttgcccctcagctttgcaaagagccaccctaggccccagctgaccgcatgggtgtgagccagcttgagaacactaactactcaataaaagcgaaggtggacatgaaaaaaaaaaaaaaaaaaa

SEQ ID NO: 67 - protein, 748 aa, Homo sapiens
MKTSPRRPLILKRRRLPLPVQNAPSETSEEEPKRSPAQQESNQAEASKEVAESNSCKFPAGIKIINHPTMPNTQVVAIPNNANIHSIITALTAKGKESGSSGPNKFILISCGGAPTQPPGLRPQTQTSYDAKRTEVTLETLGPKPAARDVNLPRPPGALCEQKRETCADGEAAGCTINNSLSNIQWLRKMSSDGLGSRSIKQEMEEKENCHLEQRQVKVEEPSRPSASWQNSVSERPPYSYMAMIQFAINSTERKRMTLKDIYTWIEDHFPYFKHIAKPGWKNSIRHNLSLHDMFVRETSANGKVSFWTIHPSANRYLTLDQVFKQQKRPNPELRRNMTIKTELPLGARRKMKPLLPRVSSYLVPIQFPVNQSLVLQPSVKVPLPLAASLMSSELARHSKRVRIAPKVLLAEEGIAPLSSAGPGKEEKLLFGEGFSPLLPVQTIKEEEIQPGEEMPHLARPIKVESPPLEEWPSPAPSFKEESSHSWEDSSQSPTPRPKKSYSGLRSPTRCVSEMLVIQHRERRERSRSRRKQHLLPPCVDEPELLFSEGPSTSRWAAELPFPADSSDPASQLSYSQEVGGPFKTPIKETLPISSTPSKSVLPRTPESWRLTPPAKVGGLDFSPVQTSQGASDPLPDPLGLMDLSTTPLQSAPPLESPQRLLSSEPLDLISVPFGNSSPSDIDVPKPGSPEPQVSGLAANRSLTEGLVLDTMNDSLSKILLDISFPGLDEDPLGPDNINWSQFIPELQ

SEQ ID NO: 68 - DNA, 3506 bp, Homo sapiens
  CDS (284)..(2530)
tttcaaacagcggaacaaactgaaagctccggtgccagaccccacccccggccccggcccgggaccccctcccctcccgggatcccccggggttcccaccccgcccgcaccgccggggacccggccggtccggcgcgagcccccgtccggggccctggctcggcccccaggttggaggagcccggagcccgccttcggagctacggcctaacggcggcggcgactgcagtctggagggtccacacttgtgattctcaatggagagtgaaaacgcagattcataatgaaaactagcccccgtcggccactgattctcaaaagacggaggctgccccttcctgttcaaaatgccccaagtgaaacatcagaggaggaacctaagagatcccctgcccaacaggagtctaatcaagcagaggcctccaaggaagtggcagagtccaactcttgcaagtttccagctgggatcaagattattaaccaccccaccatgcccaacacgcaagtagtggccatccccaacaatgctaatattcacagcatcatcacagcactgactgccaagggaaaagagagtggcagtagtgggcccaacaaattcatcctcatcagctgtgggggagccccaactcagcctccaggactccggcctcaaacccaaaccagctatgatgccaaaaggacagaagtgaccctggagaccttgggaccaaaacctgcagctagggatgtgaatcttcctagaccacctggagccctttgcgagcagaaacgggagacctgtgatggtgaggcagcaggctgcactatcaacaatagcctatccaacatccagtggcttcgaaagatgagttctgatggactgggctcccgcagcatcaagcaagagatggaggaaaaggagaattgtcacctggagcagcgacaggttaaggttgaggagccttcgagaccatcagcgtcctggcagaactctgtgtctgagcggccaccctactcttacatggccatgatacaattcgccatcaacagcactgagaggaagcgcatgactttgaaagacatctatacgtggattgaggaccactttccctactttaagcacattgccaagccaggctggaagaactccatccgccacaacctttccctgcacgacatgtttgtccgggagacgtctgccaatggcaaggtctccttctggaccattcaccccagtgccaaccgctacttgacattggaccaggtgtttaagcagcagcagaaacgaccgaatccagagctccgccggaacatgaccatcaaaaccgaactccccctgggcgcacggcggaagatgaagccactgctaccacgggtcagctcatacctggtacctatccagttcccggtgaaccagtcactggtgttgcagccctcggtgaaggtgccattgcccctggcggcttccctcatgagctcagagcttgcccgccatagcaagcgagtccgcattgcccccaaggtgctgctagctgaggaggggatagctcctctttcttctgcaggaccagggaaagaggagaaactcctgtttggagaagggttttctcctttgcttccagttcagactatcaaggaggaagaaatccagcctggggaggaaatgccacacttagcgagacccatcaaagtggagagccctcccttggaagagtggccctccccggccccatctttcaaagaggaatcatctcactcctgggaggattcgtcccaatctcccaccccaagacccaagaagtcctacagtgggcttaggtccccaacccggtgtgtctcggaaatgcttgtgattcaacacagggagaggagggagaggagccggtctcggaggaaacagcatctactgcctccctgtgtggatgagccggagctgctcttctcagaggggcccagtacttcccgctgggccgcagagctcccgttcccagcagactcctctgaccctgcctcccagctcagctactcccaggaagtgggaggaccttttaagacacccattaaggaaacgctgcccatctcctccaccccgagcaaatctgtcctccccagaacccctgaatcctggaggctcacgcccccagccaaagtagggggactggatttcagcccagtacaaacctcccagggtgcctctgaccccttgcctgaccccctggggctgatggatctcagcaccactcccttgcaaagtgctcccccccttgaatcaccgcaaaggctcctcagttcagaacccttagacctcatctccgtcccctttggcaactcttctccctcagatatagacgtccccaagccaggctccccggagccacaggtttctggccttgcagccaatcgttctctgacagaaggcctggtcctggacacaatgaatgacagcctcagcaagatcctgctggacatcagctttcctggcctggacgaggacccactgggccctgacaacatcaactggtcccagtttattcctgagctacagtagagccctgcccttgcccctgtgctcaagctgtccaccatcccgggcactccaaggctcagtgcaccccaagcctctgagtgaggacagcaggcagggactgttctgctcctcatagctccctgctgcctgattatgcaaaagtagcagtcacaccctagccactgctgggaccttgtgttccccaagagtatctgattcctctgctgtccctgccaggagctgaagggtgggaacaacaaaggcaatggtgaaaagagattaggaaccccccagcctgtttccattctctgcccagcagtctcttaccttccctgatctttgcagggtggtccgtgtaaatagtataaattctccaaattatcctctaattataaatgtaagcttatttccttagatcattatccagagactgccagaaggtgggtaggatgacctggggtttcaattgacttctgttccttgcttttagttttgatagaagggaagacctgcagtgcacggtttcttccaggctgaggtacctggatcttgggttcttcactgcagggacccagacaagtggatctgcttgccagagtcctttttgcccctccctgccacctccccgtgtttccaagtcagctttcctgcaagaagaaatcctggttaaaaaagtcttttgtattgggtcaggagttgaatttggggtgggaggatggatgcaactgaagcagagtgtgggtgcccagatgtgcgctattagatgtttctctgataatgtccccaatcataccagggagactggcattgacgagaactcaggtggaggcttgagaaggccgaaagggcccctgacctgcctggcttccttagcttgcccctcagctttgcaaagagccaccctaggccccagctgaccgcatgggtgtgagccagcttgagaacactaactactcaataaaagcgaaggtggacatgaaaaaaaaaaaaaaaaaaa

SEQ ID NO: 69 - protein, 748 aa, Homo sapiens
MKTSPRRPLILKRRRLPLPVQNAPSETSEEEPKRSPAQQESNQAEASKEVAESNSCKFPAGIKIINHPTMPNTQVVAIPNNANIHSIITALTAKGKESGSSGPNKFILISCGGAPTQPPGLRPQTQTSYDAKRTEVTLETLGPKPAARDVNLPRPPGALCEQKRETCDGEAAGCTINNSLSNIQWLRKMSSDGLGSRSIKQEMEEKENCHLEQRQVKVEEPSRPSASWQNSVSERPPYSYMAMIQFAINSTERKRMTLKDIYTWIEDHFPYFKHIAKPGWKNSIRHNLSLHDMFVRETSANGKVSFWTIHPSANRYLTLDQVFKQQQKRPNPELRRNMTIKTELPLGARRKMKPLLPRVSSYLVPIQFPVNQSLVLQPSVKVPLPLAASLMSSELARHSKRVRIAPKVLLAEEGIAPLSSAGPGKEEKLLFGEGFSPLLPVQTIKEEEIQPGEEMPHLARPIKVESPPLEEWPSPAPSFKEESSHSWEDSSQSPTPRPKKSYSGLRSPTRCVSEMLVIQHRERRERSRSRRKQHLLPPCVDEPELLFSEGPSTSRWAAELPFPADSSDPASQLSYSQEVGGPFKTPIKETLPISSTPSKSVLPRTPESWRLTPPAKVGGLDFSPVQTSQGASDPLPDPLGLMDLSTTPLQSAPPLESPQRLLSSEPLDLISVPFGNSSPSDIDVPKPGSPEPQVSGLAANRSLTEGLVLDTMNDSLSKILLDISFPGLDEDPLGPDNINWSQFIPELQ

SEQ ID NO: 70 - DNA, 3503 bp, Homo sapiens
  CDS (284)..(2527)
tttcaaacagcggaacaaactgaaagctccggtgccagaccccacccccggccccggcccgggaccccctcccctcccgggatcccccggggttcccaccccgcccgcaccgccggggacccggccggtccggcgcgagcccccgtccggggccctggctcggcccccaggttggaggagcccggagcccgccttcggagctacggcctaacggcggcggcgactgcagtctggagggtccacacttgtgattctcaatggagagtgaaaacgcagattcataatgaaaactagcccccgtcggccactgattctcaaaagacggaggctgccccttcctgttcaaaatgccccaagtgaaacatcagaggaggaacctaagagatcccctgcccaacaggagtctaatcaagcagaggcctccaaggaagtggcagagtccaactcttgcaagtttccagctgggatcaagattattaaccaccccaccatgcccaacacgcaagtagtggccatccccaacaatgctaatattcacagcatcatcacagcactgactgccaagggaaaagagagtggcagtagtgggcccaacaaattcatcctcatcagctgtgggggagccccaactcagcctccaggactccggcctcaaacccaaaccagctatgatgccaaaaggacagaagtgaccctggagaccttgggaccaaaacctgcagctagggatgtgaatcttcctagaccacctggagccctttgcgagcagaaacgggagacctgtgatggtgaggcagcaggctgcactatcaacaatagcctatccaacatccagtggcttcgaaagatgagttctgatggactgggctcccgcagcatcaagcaagagatggaggaaaaggagaattgtcacctggagcagcgacaggttaaggttgaggagccttcgagaccatcagcgtcctggcagaactctgtgtctgagcggccaccctactcttacatggccatgatacaattcgccatcaacagcactgagaggaagcgcatgactttgaaagacatctatacgtggattgaggaccactttccctactttaagcacattgccaagccaggctggaagaactccatccgccacaacctttccctgcacgacatgtttgtccgggagacgtctgccaatggcaaggtctccttctggaccattcaccccagtgccaaccgctacttgacattggaccaggtgtttaagcagcagaaacgaccgaatccagagctccgccggaacatgaccatcaaaaccgaactccccctgggcgcacggcggaagatgaagccactgctaccacgggtcagctcatacctggtacctatccagttcccggtgaaccagtcactggtgttgcagccctcggtgaaggtgccattgcccctggcggcttccctcatgagctcagagcttgcccgccatagcaagcgagtccgcattgcccccaaggtgctgctagctgaggaggggatagctcctctttcttctgcaggaccagggaaagaggagaaactcctgtttggagaagggttttctcctttgcttccagttcagactatcaaggaggaagaaatccagcctggggaggaaatgccacacttagcgagacccatcaaagtggagagccctcccttggaagagtggccctccccggccccatctttcaaagaggaatcatctcactcctgggaggattcgtcccaatctcccaccccaagacccaagaagtcctacagtgggcttaggtccccaacccggtgtgtctcggaaatgcttgtgattcaacacagggagaggagggagaggagccggtctcggaggaaacagcatctactgcctccctgtgtggatgagccggagctgctcttctcagaggggcccagtacttcccgctgggccgcagagctcccgttcccagcagactcctctgaccctgcctcccagctcagctactcccaggaagtgggaggaccttttaagacacccattaaggaaacgctgcccatctcctccaccccgagcaaatctgtcctccccagaacccctgaatcctggaggctcacgcccccagccaaagtagggggactggatttcagcccagtacaaacctcccagggtgcctctgaccccttgcctgaccccctggggctgatggatctcagcaccactcccttgcaaagtgctcccccccttgaatcaccgcaaaggctcctcagttcagaacccttagacctcatctccgtcccctttggcaactcttctccctcagatatagacgtccccaagccaggctccccggagccacaggtttctggccttgcagccaatcgttctctgacagaaggcctggtcctggacacaatgaatgacagcctcagcaagatcctgctggacatcagctttcctggcctggacgaggacccactgggccctgacaacatcaactggtcccagtttattcctgagctacagtagagccctgcccttgcccctgtgctcaagctgtccaccatcccgggcactccaaggctcagtgcaccccaagcctctgagtgaggacagcaggcagggactgttctgctcctcatagctccctgctgcctgattatgcaaaagtagcagtcacaccctagccactgctgggaccttgtgttccccaagagtatctgattcctctgctgtccctgccaggagctgaagggtgggaacaacaaaggcaatggtgaaaagagattaggaaccccccagcctgtttccattctctgcccagcagtctcttaccttccctgatctttgcagggtggtccgtgtaaatagtataaattctccaaattatcctctaattataaatgtaagcttatttccttagatcattatccagagactgccagaaggtgggtaggatgacctggggtttcaattgacttctgttccttgcttttagttttgatagaagggaagacctgcagtgcacggtttcttccaggctgaggtacctggatcttgggttcttcactgcagggacccagacaagtggatctgcttgccagagtcctttttgcccctccctgccacctccccgtgtttccaagtcagctttcctgcaagaagaaatcctggttaaaaaagtcttttgtattgggtcaggagttgaatttggggtgggaggatggatgcaactgaagcagagtgtgggtgcccagatgtgcgctattagatgtttctctgataatgtccccaatcataccagggagactggcattgacgagaactcaggtggaggcttgagaaggccgaaagggcccctgacctgcctggcttccttagcttgcccctcagctttgcaaagagccaccctaggccccagctgaccgcatgggtgtgagccagcttgagaacactaactactcaataaaagcgaaggtggacatgaaaaaaaaaaaaaaaaaaa

SEQ ID NO: 71 - protein, 747 aa, Homo sapiens
MKTSPRRPLILKRRRLPLPVQNAPSETSEEEPKRSPAQQESNQAEASKEVAESNSCKFPAGIKIINHPTMPNTQVVAIPNNANIHSIITALTAKGKESGSSGPNKFILISCGGAPTQPPGLRPQTQTSYDAKRTEVTLETLGPKPAARDVNLPRPPGALCEQKRETCDGEAAGCTINNSLSNIQWLRKMSSDGLGSRSIKQEMEEKENCHLEQRQVKVEEPSRPSASWQNSVSERPPYSYMAMIQFAINSTERKRMTLKDIYTWIEDHFPYFKHIAKPGWKNSIRHNLSLHDMFVRETSANGKVSFWTIHPSANRYLTLDQVFKQQKRPNPELRRNMTIKTELPLGARRKMKPLLPRVSSYLVPIQFPVNQSLVLQPSVKVPLPLAASLMSSELARHSKRVRIAPKVLLAEEGIAPLSSAGPGKEEKLLFGEGFSPLLPVQTIKEEEIQPGEEMPHLARPIKVESPPLEEWPSPAPSFKEESSHSWEDSSQSPTPRPKKSYSGLRSPTRCVSEMLVIQHRERRERSRSRRKQHLLPPCVDEPELLFSEGPSTSRWAAELPFPADSSDPASQLSYSQEVGGPFKTPIKETLPISSTPSKSVLPRTPESWRLTPPAKVGGLDFSPVQTSQGASDPLPDPLGLMDLSTTPLQSAPPLESPQRLLSSEPLDLISVPFGNSSPSDIDVPKPGSPEPQVSGLAANRSLTEGLVLDTMNDSLSKILLDISFPGLDEDPLGPDNINWSQFIPELQ

SEQ ID NO: 72 - DNA, 3551 bp, Homo sapiens
  CDS (284)..(2575)
tttcaaacagcggaacaaactgaaagctccggtgccagaccccacccccggccccggcccgggaccccctcccctcccgggatcccccggggttcccaccccgcccgcaccgccggggacccggccggtccggcgcgagcccccgtccggggccctggctcggcccccaggttggaggagcccggagcccgccttcggagctacggcctaacggcggcggcgactgcagtctggagggtccacacttgtgattctcaatggagagtgaaaacgcagattcataatgaaaactagcccccgtcggccactgattctcaaaagacggaggctgccccttcctgttcaaaatgccccaagtgaaacatcagaggaggaacctaagagatcccctgcccaacaggagtctaatcaagcagaggcctccaaggaagtggcagagtccaactcttgcaagtttccagctgggatcaagattattaaccaccccaccatgcccaacacgcaagtagtggccatccccaacaatgctaatattcacagcatcatcacagcactgactgccaagggaaaagagagtggcagtagtgggcccaacaaattcatcctcatcagctgtgggggagccccaactcagcctccaggactccggcctcaaacccaaaccagctatgatgccaaaaggacagaagtgaccctggagaccttgggaccaaaacctgcagctagggatgtgaatcttcctagaccacctggagccctttgcgagcagaaacgggagacctgtgcagatggtgaggcagcaggctgcactatcaacaatagcctatccaacatccagtggcttcgaaagatgagttctgatggactgggctcccgcagcatcaagcaagagatggaggaaaaggagaattgtcacctggagcagcgacaggttaaggttgaggagccttcgagaccatcagcgtcctggcagaactctgtgtctgagcggccaccctactcttacatggccatgatacaattcgccatcaacagcactgagaggaagcgcatgactttgaaagacatctatacgtggattgaggaccactttccctactttaagcacattgccaagccaggctggaagaactccatccgccacaacctttccctgcacgacatgtttgtccgggagacgtctgccaatggcaaggtctccttctggaccattcaccccagtgccaaccgctacttgacattggaccaggtgtttaagccactggacccagggtctccacaattgcccgagcacttggaatcacagcagaaacgaccgaatccagagctccgccggaacatgaccatcaaaaccgaactccccctgggcgcacggcggaagatgaagccactgctaccacgggtcagctcatacctggtacctatccagttcccggtgaaccagtcactggtgttgcagccctcggtgaaggtgccattgcccctggcggcttccctcatgagctcagagcttgcccgccatagcaagcgagtccgcattgcccccaaggtgctgctagctgaggaggggatagctcctctttcttctgcaggaccagggaaagaggagaaactcctgtttggagaagggttttctcctttgcttccagttcagactatcaaggaggaagaaatccagcctggggaggaaatgccacacttagcgagacccatcaaagtggagagccctcccttggaagagtggccctccccggccccatctttcaaagaggaatcatctcactcctgggaggattcgtcccaatctcccaccccaagacccaagaagtcctacagtgggcttaggtccccaacccggtgtgtctcggaaatgcttgtgattcaacacagggagaggagggagaggagccggtctcggaggaaacagcatctactgcctccctgtgtggatgagccggagctgctcttctcagaggggcccagtacttcccgctgggccgcagagctcccgttcccagcagactcctctgaccctgcctcccagctcagctactcccaggaagtgggaggaccttttaagacacccattaaggaaacgctgcccatctcctccaccccgagcaaatctgtcctccccagaacccctgaatcctggaggctcacgcccccagccaaagtagggggactggatttcagcccagtacaaacctcccagggtgcctctgaccccttgcctgaccccctggggctgatggatctcagcaccactcccttgcaaagtgctcccccccttgaatcaccgcaaaggctcctcagttcagaacccttagacctcatctccgtcccctttggcaactcttctccctcagatatagacgtccccaagccaggctccccggagccacaggtttctggccttgcagccaatcgttctctgacagaaggcctggtcctggacacaatgaatgacagcctcagcaagatcctgctggacatcagctttcctggcctggacgaggacccactgggccctgacaacatcaactggtcccagtttattcctgagctacagtagagccctgcccttgcccctgtgctcaagctgtccaccatcccgggcactccaaggctcagtgcaccccaagcctctgagtgaggacagcaggcagggactgttctgctcctcatagctccctgctgcctgattatgcaaaagtagcagtcacaccctagccactgctgggaccttgtgttccccaagagtatctgattcctctgctgtccctgccaggagctgaagggtgggaacaacaaaggcaatggtgaaaagagattaggaaccccccagcctgtttccattctctgcccagcagtctcttaccttccctgatctttgcagggtggtccgtgtaaatagtataaattctccaaattatcctctaattataaatgtaagcttatttccttagatcattatccagagactgccagaaggtgggtaggatgacctggggtttcaattgacttctgttccttgcttttagttttgatagaagggaagacctgcagtgcacggtttcttccaggctgaggtacctggatcttgggttcttcactgcagggacccagacaagtggatctgcttgccagagtcctttttgcccctccctgccacctccccgtgtttccaagtcagctttcctgcaagaagaaatcctggttaaaaaagtcttttgtattgggtcaggagttgaatttggggtgggaggatggatgcaactgaagcagagtgtgggtgcccagatgtgcgctattagatgtttctctgataatgtccccaatcataccagggagactggcattgacgagaactcaggtggaggcttgagaaggccgaaagggcccctgacctgcctggcttccttagcttgcccctcagctttgcaaagagccaccctaggccccagctgaccgcatgggtgtgagccagcttgagaacactaactactcaataaaagcgaaggtggacatgaaaaaaaaaaaaaaaaaaa

SEQ ID NO: 73 - protein, 763 aa, Homo sapiens
MKTSPRRPLILKRRRLPLPVQNAPSETSEEEPKRSPAQQESNQAEASKEVAESNSCKFPAGIKIINHPTMPNTQVVAIPNNANIHSIITALTAKGKESGSSGPNKFILISCGGAPTQPPGLRPQTQTSYDAKRTEVTLETLGPKPAARDVNLPRPPGALCEQKRETCADGEAAGCTINNSLSNIQWLRKMSSDGLGSRSIKQEMEEKENCHLEQRQVKVEEPSRPSASWQNSVSERPPYSYMAMIQFAINSTERKRMTLKDIYTWIEDHFPYFKHIAKPGWKNSIRHNLSLHDMFVRETSANGKVSFWTIHPSANRYLTLDQVFKPLDPGSPQLPEHLESQQKRPNPELRRNMTIKTELPLGARRKMKPLLPRVSSYLVPIQFPVNQSLVLQPSVKVPLPLAASLMSSELARHSKRVRIAPKVLLAEEGIAPLSSAGPGKEEKLLFGEGFSPLLPVQTIKEEEIQPGEEMPHLARPIKVESPPLEEWPSPAPSFKEESSHSWEDSSQSPTPRPKKSYSGLRSPTRCVSEMLVIQHRERRERSRSRRKQHLLPPCVDEPELLFSEGPSTSRWAAELPFPADSSDPASQLSYSQEVGGPFKTPIKETLPISSTPSKSVLPRTPESWRLTPPAKVGGLDFSPVQTSQGASDPLPDPLGLMDLSTTPLQSAPPLESPQRLLSSEPLDLISVPFGNSSPSDIDVPKPGSPEPQVSGLAANRSLTEGLVLDTMNDSLSKILLDISFPGLDEDPLGPDNINWSQFIPELQ

SEQ ID NO: 74 - DNA, 3665 bp, Homo sapiens
  CDS (284)..(2689)
tttcaaacagcggaacaaactgaaagctccggtgccagaccccacccccggccccggcccgggaccccctcccctcccgggatcccccggggttcccaccccgcccgcaccgccggggacccggccggtccggcgcgagcccccgtccggggccctggctcggcccccaggttggaggagcccggagcccgccttcggagctacggcctaacggcggcggcgactgcagtctggagggtccacacttgtgattctcaatggagagtgaaaacgcagattcataatgaaaactagcccccgtcggccactgattctcaaaagacggaggctgccccttcctgttcaaaatgccccaagtgaaacatcagaggaggaacctaagagatcccctgcccaacaggagtctaatcaagcagaggcctccaaggaagtggcagagtccaactcttgcaagtttccagctgggatcaagattattaaccaccccaccatgcccaacacgcaagtagtggccatccccaacaatgctaatattcacagcatcatcacagcactgactgccaagggaaaagagagtggcagtagtgggcccaacaaattcatcctcatcagctgtgggggagccccaactcagcctccaggactccggcctcaaacccaaaccagctatgatgccaaaaggacagaagtgaccctggagaccttgggaccaaaacctgcagctagggatgtgaatcttcctagaccacctggagccctttgcgagcagaaacgggagacctgtgcagatggtgaggcagcaggctgcactatcaacaatagcctatccaacatccagtggcttcgaaagatgagttctgatggactgggctcccgcagcatcaagcaagagatggaggaaaaggagaattgtcacctggagcagcgacaggttaaggttgaggagccttcgagaccatcagcgtcctggcagaactctgtgtctgagcggccaccctactcttacatggccatgatacaattcgccatcaacagcactgagaggaagcgcatgactttgaaagacatctatacgtggattgaggaccactttccctactttaagcacattgccaagccaggctggaagaactccatccgccacaacctttccctgcacgacatgtttgtccgggagacgtctgccaatggcaaggtctccttctggaccattcaccccagtgccaaccgctacttgacattggaccaggtgtttaagccactggacccagggtctccacaattgcccgagcacttggaatcacagcagaaacgaccgaatccagagctccgccggaacatgaccatcaaaaccgaactccccctgggcgcacggcggaagatgaagccactgctaccacgggtcagctcatacctggtacctatccagttcccggtgaaccagtcactggtgttgcagccctcggtgaaggtgccattgcccctggcggcttccctcatgagctcagagcttgcccgccatagcaagcgagtccgcattgcccccaaggtttttggggaacaggtggtgtttggttacatgagtaagttctttagtggcgatctgcgagattttggtacacccatcaccagcttgtttaattttatctttctttgtttatcagtgctgctagctgaggaggggatagctcctctttcttctgcaggaccagggaaagaggagaaactcctgtttggagaagggttttctcctttgcttccagttcagactatcaaggaggaagaaatccagcctggggaggaaatgccacacttagcgagacccatcaaagtggagagccctcccttggaagagtggccctccccggccccatctttcaaagaggaatcatctcactcctgggaggattcgtcccaatctcccaccccaagacccaagaagtcctacagtgggcttaggtccccaacccggtgtgtctcggaaatgcttgtgattcaacacagggagaggagggagaggagccggtctcggaggaaacagcatctactgcctccctgtgtggatgagccggagctgctcttctcagaggggcccagtacttcccgctgggccgcagagctcccgttcccagcagactcctctgaccctgcctcccagctcagctactcccaggaagtgggaggaccttttaagacacccattaaggaaacgctgcccatctcctccaccccgagcaaatctgtcctccccagaacccctgaatcctggaggctcacgcccccagccaaagtagggggactggatttcagcccagtacaaacctcccagggtgcctctgaccccttgcctgaccccctggggctgatggatctcagcaccactcccttgcaaagtgctcccccccttgaatcaccgcaaaggctcctcagttcagaacccttagacctcatctccgtcccctttggcaactcttctccctcagatatagacgtccccaagccaggctccccggagccacaggtttctggccttgcagccaatcgttctctgacagaaggcctggtcctggacacaatgaatgacagcctcagcaagatcctgctggacatcagctttcctggcctggacgaggacccactgggccctgacaacatcaactggtcccagtttattcctgagctacagtagagccctgcccttgcccctgtgctcaagctgtccaccatcccgggcactccaaggctcagtgcaccccaagcctctgagtgaggacagcaggcagggactgttctgctcctcatagctccctgctgcctgattatgcaaaagtagcagtcacaccctagccactgctgggaccttgtgttccccaagagtatctgattcctctgctgtccctgccaggagctgaagggtgggaacaacaaaggcaatggtgaaaagagattaggaaccccccagcctgtttccattctctgcccagcagtctcttaccttccctgatctttgcagggtggtccgtgtaaatagtataaattctccaaattatcctctaattataaatgtaagcttatttccttagatcattatccagagactgccagaaggtgggtaggatgacctggggtttcaattgacttctgttccttgcttttagttttgatagaagggaagacctgcagtgcacggtttcttccaggctgaggtacctggatcttgggttcttcactgcagggacccagacaagtggatctgcttgccagagtcctttttgcccctccctgccacctccccgtgtttccaagtcagctttcctgcaagaagaaatcctggttaaaaaagtcttttgtattgggtcaggagttgaatttggggtgggaggatggatgcaactgaagcagagtgtgggtgcccagatgtgcgctattagatgtttctctgataatgtccccaatcataccagggagactggcattgacgagaactcaggtggaggcttgagaaggccgaaagggcccctgacctgcctggcttccttagcttgcccctcagctttgcaaagagccaccctaggccccagctgaccgcatgggtgtgagccagcttgagaacactaactactcaataaaagcgaaggtggacatgaaaaaaaaaaaaaaaaaaa

SEQ ID NO: 75 - protein, 801 aa, Homo sapiens
MKTSPRRPLILKRRRLPLPVQNAPSETSEEEPKRSPAQQESNQAEASKEVAESNSCKFPAGIKIINHPTMPNTQVVAIPNNANIHSIITALTAKGKESGSSGPNKFILISCGGAPTQPPGLRPQTQTSYDAKRTEVTLETLGPKPAARDVNLPRPPGALCEQKRETCADGEAAGCTINNSLSNIQWLRKMSSDGLGSRSIKQEMEEKENCHLEQRQVKVEEPSRPSASWQNSVSERPPYSYMAMIQFAINSTERKRMTLKDIYTWIEDHFPYFKHIAKPGWKNSIRHNLSLHDMFVRETSANGKVSFWTIHPSANRYLTLDQVFKPLDPGSPQLPEHLESQQKRPNPELRRNMTIKTELPLGARRKMKPLLPRVSSYLVPIQFPVNQSLVLQPSVKVPLPLAASLMSSELARHSKRVRIAPKVFGEQVVFGYMSKFFSGDLRDFGTPITSLFNFIFLCLSVLLAEEGIAPLSSAGPGKEEKLLFGEGFSPLLPVQTIKEEEIQPGEEMPHLARPIKVESPPLEEWPSPAPSFKEESSHSWEDSSQSPTPRPKKSYSGLRSPTRCVSEMLVIQHRERRERSRSRRKQHLLPPCVDEPELLFSEGPSTSRWAAELPFPADSSDPASQLSYSQEVGGPFKTPIKETLPISSTPSKSVLPRTPESWRLTPPAKVGGLDFSPVQTSQGASDPLPDPLGLMDLSTTPLQSAPPLESPQRLLSSEPLDLISVPFGNSSPSDIDVPKPGSPEPQVSGLAANRSLTEGLVLDTMNDSLSKILLDISFPGLDEDPLGPDNINWSQFIPELQ

SEQ ID NO: 76 - protein, 4 aa, Artificial Sequence
  a linker peptide
NKRK